European Patent Application EP 4 144 765 A1, published March 8, 2023. Title: DETECTION REAGENT FOR SCREENING BLOCKING AGENT OF CORONAVIRUS INFECTIONS, AND DETECTION METHOD. Applicant: YANG SHENG TANG COMPANY, LTD. XIAMEN UNIVERSITY. The sequence listing filed with the application follows.

SEQUENCE LISTING (42 sequences)

SEQ ID NO: 1 - protein, 235 aa, Artificial sequence
  SARS-CoV-2-RBD amino acid sequence
SNFRVQPTESIVRFPNITNLCPFGEVFNATRFASVYAWNRKRISNCVADYSVLYNSASFSTFKCYGVSPTKLNDLCFTNVYADSFVIRGDEVRQIAPGQTGKIADYNYKLPDDFTGCVIAWNSNNLDSKVGGNYNYLYRLFRKSNLKPFERDISTEIYQAGSTPCNGVEGFNCYFPLQSYGFQPTNGVGYQPYRVVVLSFELLHAPATVCGPKKSTNLVKNKCVNFNFNGLTGTG

SEQ ID NO: 2 - DNA, 705 bp, Artificial sequence
  SARS-CoV-2-RBD nucleic acid sequence
agcaacttccgcgtgcagcccaccgagagcatcgtgcgcttccccaacatcaccaacctgtgccccttcggcgaggtgttcaacgccacccgcttcgccagcgtgtacgcctggaaccgcaagcgcatcagcaactgcgtggccgactacagcgtgctgtacaacagcgccagcttcagcaccttcaagtgctacggcgtgagccccaccaagctgaacgacctgtgcttcaccaacgtgtacgccgacagcttcgtgatccgcggcgacgaggtgcgccagatcgcccccggccagaccggcaagatcgccgactacaactacaagctgcccgacgacttcaccggctgcgtgatcgcctggaacagcaacaacctggacagcaaggtgggcggcaactacaactacctgtaccgcctgttccgcaagagcaacctgaagcccttcgagcgcgacatcagcaccgagatataccaggccggcagcaccccctgcaacggcgtggagggcttcaactgctacttccccctgcagagctacggcttccagcccaccaacggcgtgggctaccagccctaccgcgtggtggtgctgagcttcgagctgctgcacgcccccgccaccgtgtgcggccccaagaagagcaccaacctggtgaagaacaagtgcgtgaacttcaacttcaacggcctgaccggcaccggc

SEQ ID NO: 3 - DNA, 60 bp, Artificial sequence
  B2M signal peptide nucleic acid sequence
atggcccgcagcgtgaccctggtgttcctggtgctggtgagcctgaccggtctgtacgcc

SEQ ID NO: 4 - DNA, 714 bp, Artificial sequence
  Green fluorescent protein mGamillus nucleic acid sequence
gtgagcaagggcgaggaggcatctggcagagccctgttccagtaccccatgaccagcaagatcgagctgaacggcgagatcaacggcaagaaattcaaggtggccggcgagggcttcacccccagcagcggcagattcaacatgcacgcctactgcaccaccggcgacctgcctatgagctgggtcgtgattgccagccccctccagtacggcttccacatgttcgcccactaccccgaggacatcacacactttttccaggaatgcttccccggcagctacaccctggaccggaccctgagaatggaaggcgacggcaccctgaccacccaccacgagtacagcctggaggacggctgcgtgacctccaagaccaccctgaatgccagcggcttcgaccctaagggcgccaccatgaccaagagcttcgtgaaacaactgcctaacgaggtgaagatcaccccccacggccccaacggcatcagactgaccagcaccgtgctgtacctgaaggaggatggcaccatccagatcggcacccaggactgcatcgtgacccctgtgggcggaaggaaagtgacccagcccaaggcccacttcctgcacacccagatcatccagaagaaggaccccaacgacacccgggaccacatcgtgcagacagaactggccgtggccggcaatctgtggcacggcatggacgagctgtacaag

SEQ ID NO: 5 - DNA, 705 bp, Artificial sequence
  Green fluorescent protein mNeonGreen nucleic acid sequence
gtgagcaagggcgaggaggacaacatggccagcctgcccgccacccacgagctgcacatcttcggcagcatcaacggcgtggacttcgacatggtgggccagggcaccggcaaccccaacgacggctacgaggagctgaacctgaagagcaccaagggcgacctgcagttcagcccctggatcttagtgccccacatcggctacggcttccaccagtacctgccctaccccgacggcatgagccccttccaggccgccatggtggacggcagcggctaccaggtgcaccgcaccatgcagttcgaggacggcgccagcctgaccgtgaactaccgctacacctacgagggcagccacatcaagggcgaggcccaggtgaagggcaccggcttccccgccgacggccccgtgatgaccaacagcctgaccgccgccgactggtgccgcagcaagaagacctaccccaacgacaagaccatcatcagcaccttcaagtggagctacaccaccggcaacggcaagcgctaccgcagcaccgcccgcaccacctacaccttcgccaagcccatggccgccaactacctgaagaaccagcccatgtacgtgttccgcaagaccgagctgaagcacagcaagaccgagctgaacttcaaggagtggcagaaggccttcaccgacgtgatgggcatggacgagctgtacaag

SEQ ID NO: 6 - protein, 20 aa, Artificial sequence
  Flexible amino acid linker sequence amino acid sequence
GGGGSGGGGSGGGGSGGGGS

SEQ ID NO: 7 - protein, 525 aa, Artificial sequence
  SARS-CoV2-RBG amino acid sequence
MARSVTLVFLVLVSLTGLYASNFRVQPTESIVRFPNITNLCPFGEVFNATRFASVYAWNRKRISNCVADYSVLYNSASFSTFKCYGVSPTKLNDLCFTNVYADSFVIRGDEVRQIAPGQTGKIADYNYKLPDDFTGCVIAWNSNNLDSKVGGNYNYLYRLFRKSNLKPFERDISTEIYQAGSTPCNGVEGFNCYFPLQSYGFQPTNGVGYQPYRVVVLSFELLHAPATVCGPKKSTNLVKNKCVNFNFNGLTGTGRSGGGGSGGGGSGGGGSGGGGSGVSKGEEASGRALFQYPMTSKIELNGEINGKKFKVAGEGFTPSSGRFNMHAYCTTGDLPMSWVVIASPLQYGFHMFAHYPEDITHFFQECFPGSYTLDRTLRMEGDGTLTTHHEYSLEDGCVTSKTTLNASGFDPKGATMTKSFVKQLPNEVKITPHGPNGIRLTSTVLYLKEDGTIQIGTQDCIVTPVGGRKVTQPKAHFLHTQIIQKKDPNDTRDHIVQTELAVAGNLWHGMDELYKGSGHHHHHH

SEQ ID NO: 8 - protein, 525 aa, Artificial sequence
  SARS-CoV2-RBN amino acid sequence
MARSVTLVFLVLVSLTGLYASNFRVQPTESIVRFPNITNLCPFGEVFNATRFASVYAWNRKRISNCVADYSVLYNSASFSTFKCYGVSPTKLNDLCFTNVYADSFVIRGDEVRQIAPGQTGKIADYNYKLPDDFTGCVIAWNSNNLDSKVGGNYNYLYRLFRKSNLKPFERDISTEIYQAGSTPCNGVEGFNCYFPLQSYGFQPTNGVGYQPYRVVVLSFELLHAPATVCGPKKSTNLVKNKCVNFNFNGLTGTGSASGGGGSGGGGSGGGGSGGGGSGVSKGEEDNMASLPATHELHIFGSINGVDFDMVGQGTGNPNDGYEELNLKSTKGDLQFSPWILVPHIGYGFHQYLPYPDGMSPFQAAMVDGSGYQVHRTMQFEDGASLTVNYRYTYEGSHIKGEAQVKGTGFPADGPVMTNSLTAADWCRSKKTYPNDKTIISTFKWSYTTGNGKRYRSTARTTYTFAKPMAANYLKNQPMYVFRKTELKHSKTELNFKEWQKAFTDVMGMDELYKSLEHHHHHHHH

SEQ ID NO: 9 - DNA, 1578 bp, Artificial sequence
  SARS-CoV2-RBG nucleic acid sequence
atggcccgcagcgtgaccctggtgttcctggtgctggtgagcctgaccggtctgtacgccagcaacttccgcgtgcagcccaccgagagcatcgtgcgcttccccaacatcaccaacctgtgccccttcggcgaggtgttcaacgccacccgcttcgccagcgtgtacgcctggaaccgcaagcgcatcagcaactgcgtggccgactacagcgtgctgtacaacagcgccagcttcagcaccttcaagtgctacggcgtgagccccaccaagctgaacgacctgtgcttcaccaacgtgtacgccgacagcttcgtgatccgcggcgacgaggtgcgccagatcgcccccggccagaccggcaagatcgccgactacaactacaagctgcccgacgacttcaccggctgcgtgatcgcctggaacagcaacaacctggacagcaaggtgggcggcaactacaactacctgtaccgcctgttccgcaagagcaacctgaagcccttcgagcgcgacatcagcaccgagatataccaggccggcagcaccccctgcaacggcgtggagggcttcaactgctacttccccctgcagagctacggcttccagcccaccaacggcgtgggctaccagccctaccgcgtggtggtgctgagcttcgagctgctgcacgcccccgccaccgtgtgcggccccaagaagagcaccaacctggtgaagaacaagtgcgtgaacttcaacttcaacggcctgaccggcaccggcagatctggcggcggaggaagcggaggaggtggcagcggtggcggtggctccggcggaggtggatccggcgtgagcaagggcgaggaggcatctggcagagccctgttccagtaccccatgaccagcaagatcgagctgaacggcgagatcaacggcaagaaattcaaggtggccggcgagggcttcacccccagcagcggcagattcaacatgcacgcctactgcaccaccggcgacctgcctatgagctgggtcgtgattgccagccccctccagtacggcttccacatgttcgcccactaccccgaggacatcacacactttttccaggaatgcttccccggcagctacaccctggaccggaccctgagaatggaaggcgacggcaccctgaccacccaccacgagtacagcctggaggacggctgcgtgacctccaagaccaccctgaatgccagcggcttcgaccctaagggcgccaccatgaccaagagcttcgtgaaacaactgcctaacgaggtgaagatcaccccccacggccccaacggcatcagactgaccagcaccgtgctgtacctgaaggaggatggcaccatccagatcggcacccaggactgcatcgtgacccctgtgggcggaaggaaagtgacccagcccaaggcccacttcctgcacacccagatcatccagaagaaggaccccaacgacacccgggaccacatcgtgcagacagaactggccgtggccggcaatctgtggcacggcatggacgagctgtacaagggtagcggtcaccaccaccaccaccactga

SEQ ID NO: 10 - DNA, 1578 bp, Artificial sequence
  SARS-CoV2-RBN nucleic acid sequence
atggcccgcagcgtgaccctggtgttcctggtgctggtgagcctgaccggtctgtacgccagcaacttccgcgtgcagcccaccgagagcatcgtgcgcttccccaacatcaccaacctgtgccccttcggcgaggtgttcaacgccacccgcttcgccagcgtgtacgcctggaaccgcaagcgcatcagcaactgcgtggccgactacagcgtgctgtacaacagcgccagcttcagcaccttcaagtgctacggcgtgagccccaccaagctgaacgacctgtgcttcaccaacgtgtacgccgacagcttcgtgatccgcggcgacgaggtgcgccagatcgcccccggccagaccggcaagatcgccgactacaactacaagctgcccgacgacttcaccggctgcgtgatcgcctggaacagcaacaacctggacagcaaggtgggcggcaactacaactacctgtaccgcctgttccgcaagagcaacctgaagcccttcgagcgcgacatcagcaccgagatataccaggccggcagcaccccctgcaacggcgtggagggcttcaactgctacttccccctgcagagctacggcttccagcccaccaacggcgtgggctaccagccctaccgcgtggtggtgctgagcttcgagctgctgcacgcccccgccaccgtgtgcggccccaagaagagcaccaacctggtgaagaacaagtgcgtgaacttcaacttcaacggcctgaccggcaccggcagcgctagcggcggcggaggaagcggaggaggtggcagcggtggcggtggctccggcggaggtggatccggcgtgagcaagggcgaggaggacaacatggccagcctgcccgccacccacgagctgcacatcttcggcagcatcaacggcgtggacttcgacatggtgggccagggcaccggcaaccccaacgacggctacgaggagctgaacctgaagagcaccaagggcgacctgcagttcagcccctggatcttagtgccccacatcggctacggcttccaccagtacctgccctaccccgacggcatgagccccttccaggccgccatggtggacggcagcggctaccaggtgcaccgcaccatgcagttcgaggacggcgccagcctgaccgtgaactaccgctacacctacgagggcagccacatcaagggcgaggcccaggtgaagggcaccggcttccccgccgacggccccgtgatgaccaacagcctgaccgccgccgactggtgccgcagcaagaagacctaccccaacgacaagaccatcatcagcaccttcaagtggagctacaccaccggcaacggcaagcgctaccgcagcaccgcccgcaccacctacaccttcgccaagcccatggccgccaactacctgaagaaccagcccatgtacgtgttccgcaagaccgagctgaagcacagcaagaccgagctgaacttcaaggagtggcagaaggccttcaccgacgtgatgggcatggacgagctgtacaagagcctcgagcatcaccaccaccaccaccaccactaa

SEQ ID NO: 11 - DNA, 795 bp, Artificial sequence
  SARS-CoV2-RBD-His nucleic acid sequence
atggcccgcagcgtgaccctggtgttcctggtgctggtgagcctgaccggtctgtacgccagcaacttccgcgtgcagcccaccgagagcatcgtgcgcttccccaacatcaccaacctgtgccccttcggcgaggtgttcaacgccacccgcttcgccagcgtgtacgcctggaaccgcaagcgcatcagcaactgcgtggccgactacagcgtgctgtacaacagcgccagcttcagcaccttcaagtgctacggcgtgagccccaccaagctgaacgacctgtgcttcaccaacgtgtacgccgacagcttcgtgatccgcggcgacgaggtgcgccagatcgcccccggccagaccggcaagatcgccgactacaactacaagctgcccgacgacttcaccggctgcgtgatcgcctggaacagcaacaacctggacagcaaggtgggcggcaactacaactacctgtaccgcctgttccgcaagagcaacctgaagcccttcgagcgcgacatcagcaccgagatataccaggccggcagcaccccctgcaacggcgtggagggcttcaactgctacttccccctgcagagctacggcttccagcccaccaacggcgtgggctaccagccctaccgcgtggtggtgctgagcttcgagctgctgcacgcccccgccaccgtgtgcggccccaagaagagcaccaacctggtgaagaacaagtgcgtgaacttcaacttcaacggcctgaccggcaccggcagatctggtcaccaccaccaccaccactga

SEQ ID NO: 12 - protein, 264 aa, Artificial sequence
  SARS-CoV2-RBD-His amino acid sequence
MARSVTLVFLVLVSLTGLYASNFRVQPTESIVRFPNITNLCPFGEVFNATRFASVYAWNRKRISNCVADYSVLYNSASFSTFKCYGVSPTKLNDLCFTNVYADSFVIRGDEVRQIAPGQTGKIADYNYKLPDDFTGCVIAWNSNNLDSKVGGNYNYLYRLFRKSNLKPFERDISTEIYQAGSTPCNGVEGFNCYFPLQSYGFQPTNGVGYQPYRVVVLSFELLHAPATVCGPKKSTNLVKNKCVNFNFNGLTGTGRSGHHHHHH

SEQ ID NO: 13 - protein, 524 aa, Artificial sequence
  SARS-CoV1-RBG amino acid sequence
MARSVTLVFLVLVSLTGLYASNFRVVPSGDVVRFPNITNLCPFGEVFNATKFPSVYAWERKKISNCVADYSVLYNSTFFSTFKCYGVSATKLNDLCFSNVYADSFVVKGDDVRQIAPGQTGVIADYNYKLPDDFMGCVLAWNTRNIDATSTGNYNYKYRYLRHGKLRPFERDISNVPFSPDGKPCTPPALNCYWPLNDYGFYTTTGIGYQPYRVVVLSFELLNAPATVCGPKLSTDLIKNQCVNFNFNGLTGTGRSGGGGSGGGGSGGGGSGGGGSGVSKGEEASGRALFQYPMTSKIELNGEINGKKFKVAGEGFTPSSGRFNMHAYCTTGDLPMSWVVIASPLQYGFHMFAHYPEDITHFFQECFPGSYTLDRTLRMEGDGTLTTHHEYSLEDGCVTSKTTLNASGFDPKGATMTKSFVKQLPNEVKITPHGPNGIRLTSTVLYLKEDGTIQIGTQDCIVTPVGGRKVTQPKAHFLHTQIIQKKDPNDTRDHIVQTELAVAGNLWHGMDELYKGSGHHHHHH

SEQ ID NO: 14 - DNA, 1575 bp, Artificial sequence
  SARS-CoV1-RBG nucleic acid sequence
atggcccgcagcgtgaccctggtgttcctggtgctggtgagcctgaccggtctgtacgccagcaacttcagggtggtgccatctggagatgtggtgaggtttccaaacatcaccaacctgtgtccatttggagaggtgttcaatgccaccaagtttccatctgtctatgcctgggagaggaagaagattagcaactgtgtggctgactactctgtgctctacaacagcaccttcttcagcaccttcaagtgttatggagtgtctgccaccaaactgaatgacctgtgtttcagcaatgtctatgctgactcctttgtggtgaagggagatgatgtgagacagattgcccctggacaaacaggagtgattgctgactacaactacaaactgcctgatgactttatgggctgtgtgctggcttggaacaccaggaacattgatgccaccagcacaggcaactacaactacaaatacagatacctgagacatggcaaactgagaccatttgagagggacatcagcaatgtgccattcagccctgatggcaagccatgtactcctcctgccctgaactgttactggccactgaatgactatggcttctacaccaccacaggcattggctaccaaccatacagggtggtggtgctgtcctttgaactgctgaatgcccctgccacagtgtgtggaccaaaactgagcacagacctgattaagaaccagtgtgtgaacttcaacttcaatggactgacaggcacaggaagatctggcggcggaggaagcggaggaggtggcagcggtggcggtggctccggcggaggtggatccggcgtgagcaagggcgaggaggcatctggcagagccctgttccagtaccccatgaccagcaagatcgagctgaacggcgagatcaacggcaagaaattcaaggtggccggcgagggcttcacccccagcagcggcagattcaacatgcacgcctactgcaccaccggcgacctgcctatgagctgggtcgtgattgccagccccctccagtacggcttccacatgttcgcccactaccccgaggacatcacacactttttccaggaatgcttccccggcagctacaccctggaccggaccctgagaatggaaggcgacggcaccctgaccacccaccacgagtacagcctggaggacggctgcgtgacctccaagaccaccctgaatgccagcggcttcgaccctaagggcgccaccatgaccaagagcttcgtgaaacaactgcctaacgaggtgaagatcaccccccacggccccaacggcatcagactgaccagcaccgtgctgtacctgaaggaggatggcaccatccagatcggcacccaggactgcatcgtgacccctgtgggcggaaggaaagtgacccagcccaaggcccacttcctgcacacccagatcatccagaagaaggaccccaacgacacccgggaccacatcgtgcagacagaactggccgtggccggcaatctgtggcacggcatggacgagctgtacaagggtagcggtcaccaccaccaccaccactga

SEQ ID NO: 15 - protein, 542 aa, Artificial sequence
  MERS-RBG amino acid sequence
MARSVTLVFLVLVSLTGLYASSFEAKPSGSVVEQAEGVECDFSPLLSGTPPQVYNFKRLVFTNCNYNLTKLLSLFSVNDFTCSQISPAAIASNCYSSLILDYFSYPLSMKSDLSVSSAGPISQFNYKQSFSNPTCLILATVPHNLTTITKPLKYSYINKCSRLLSDDRTEVPQLVNANQYSPCVSIVPSTVWEDGDYYRKQLSPLEGGGWLVASGSTVAMTEQLQMGFGITVQYGTDTNSVCPKLEFANDTKIASQLGNCVEYSLYGVSGRGRSGGGGSGGGGSGGGGSGGGGSGVSKGEEASGRALFQYPMTSKIELNGEINGKKFKVAGEGFTPSSGRFNMHAYCTTGDLPMSWVVIASPLQYGFHMFAHYPEDITHFFQECFPGSYTLDRTLRMEGDGTLTTHHEYSLEDGCVTSKTTLNASGFDPKGATMTKSFVKQLPNEVKITPHGPNGIRLTSTVLYLKEDGTIQIGTQDCIVTPVGGRKVTQPKAHFLHTQIIQKKDPNDTRDHIVQTELAVAGNLWHGMDELYKGSGHHHHHH

SEQ ID NO: 16 - DNA, 1629 bp, Artificial sequence
  MERS-RBG nucleic acid sequence
atggcccgcagcgtgaccctggtgttcctggtgctggtgagcctgaccggtctgtacgcctcctcctttgaggctaagccatctggctctgtggtggaacaggctgagggagtggagtgtgacttcagcccactgctgtctggcacacctccacaggtctacaacttcaagagactggtgttcaccaactgtaactacaacctgaccaaactgctgtccctgttctctgtgaatgacttcacttgtagccagattagccctgctgccattgccagcaactgttactcctccctgattctggactacttctcctacccactgagtatgaagtctgacctgtctgtgtcctctgctggaccaatcagccagttcaactacaagcagtccttcagcaacccaacttgtctgattctggctacagtgccacacaacctgaccaccatcaccaagccactgaaatactcctacatcaacaagtgtagcagactgctgtctgatgacaggacagaggtgccacaactagtgaatgccaaccaatacagcccatgtgtgagcattgtgccaagcacagtgtgggaggatggagactactacaggaagcaacttagcccattggagggaggaggctggctggtggcatctggcagcacagtggctatgacagaacaactccaaatgggctttggcatcacagtccaatatggcacagacaccaactctgtgtgtccaaaattggagtttgccaatgacaccaagattgccagccaacttggcaactgtgtggaatactccctctatggagtgtctggcaggggaagatctggcggcggaggaagcggaggaggtggcagcggtggcggtggctccggcggaggtggatccggcgtgagcaagggcgaggaggcatctggcagagccctgttccagtaccccatgaccagcaagatcgagctgaacggcgagatcaacggcaagaaattcaaggtggccggcgagggcttcacccccagcagcggcagattcaacatgcacgcctactgcaccaccggcgacctgcctatgagctgggtcgtgattgccagccccctccagtacggcttccacatgttcgcccactaccccgaggacatcacacactttttccaggaatgcttccccggcagctacaccctggaccggaccctgagaatggaaggcgacggcaccctgaccacccaccacgagtacagcctggaggacggctgcgtgacctccaagaccaccctgaatgccagcggcttcgaccctaagggcgccaccatgaccaagagcttcgtgaaacaactgcctaacgaggtgaagatcaccccccacggccccaacggcatcagactgaccagcaccgtgctgtacctgaaggaggatggcaccatccagatcggcacccaggactgcatcgtgacccctgtgggcggaaggaaagtgacccagcccaaggcccacttcctgcacacccagatcatccagaagaaggaccccaacgacacccgggaccacatcgtgcagacagaactggccgtggccggcaatctgtggcacggcatggacgagctgtacaagggtagcggtcaccaccaccaccaccactga

SEQ ID NO: 17 - protein, 617 aa, Artificial sequence
  HKU1-RBG amino acid sequence
MARSVTLVFLVLVSLTGLYASGFTVKPVATVHRRIPDLPDCDIDKWLNNFNVPSPLNWERKIFSNCNFNLSTLLRLVHTDSFSCNNFDESKIYGSCFKSIVLDKFAIPNSRRSDLQLGSSGFLQSSNYKIDTTSSSCQLYYSLPAINVTINNYNPSSWNRRYGFNNFNLSSHSVVYSRYCFSVNNTFCPCAKPSFASSCKSHKPPSASCPIGTNYRSCESTTVLDHTDWCRCSCLPDPITAYDPRSCSQKKSLVGVGEHCAGFGVDEEKCGVLDGSYNVSCLCSTDAFLGWSYDTCVSNNRCNIFSNFILNGINSGTTCSNDLLQPNTEVFTDVCVDYDLYGITGQGRSGGGGSGGGGSGGGGSGGGGSGVSKGEEASGRALFQYPMTSKIELNGEINGKKFKVAGEGFTPSSGRFNMHAYCTTGDLPMSWVVIASPLQYGFHMFAHYPEDITHFFQECFPGSYTLDRTLRMEGDGTLTTHHEYSLEDGCVTSKTTLNASGFDPKGATMTKSFVKQLPNEVKITPHGPNGIRLTSTVLYLKEDGTIQIGTQDCIVTPVGGRKVTQPKAHFLHTQIIQKKDPNDTRDHIVQTELAVAGNLWHGMDELYKGSGHHHHHH

SEQ ID NO: 18 - DNA, 1854 bp, Artificial sequence
  HKU1-RBG nucleic acid sequence
atggcccgcagcgtgaccctggtgttcctggtgctggtgagcctgaccggtctgtacgcctctggcttcacagtgaagcctgtggccacagtgcacaggaggatacctgacctgcctgactgtgacattgacaagtggctgaacaacttcaatgtgccatcccccctgaactgggagaggaagatcttctccaactgcaacttcaacctgtccaccctgctgaggctggtgcacacagactccttctcctgcaacaactttgatgagtccaagatctatggctcctgcttcaagtccattgtgctggacaagtttgccatccccaactccaggaggtctgacctgcagctgggctcctctggcttcctgcagtcctccaactacaagattgacaccacctcctcctcctgccagctgtactactccctgcctgccatcaatgtgaccatcaacaactacaacccatcctcctggaacaggaggtatggcttcaacaacttcaacctgtcctcccactctgtggtctactccaggtactgcttctctgtgaacaacaccttctgcccatgtgccaagccatcctttgcctcctcctgcaagtcccacaagcccccatctgcctcctgccccattggcaccaactacaggtcctgtgagtccaccacagtgctggaccacacagactggtgcaggtgctcctgcctgcctgaccccatcacagcctatgaccccaggtcctgctcccagaagaagtccctggtgggcgtgggcgagcactgtgctggctttggcgtggatgaggagaagtgtggcgtgctggatggctcctacaatgtctcctgcctgtgctccacagatgccttcctgggctggtcctatgacacctgtgtctccaacaacaggtgcaacatcttctccaacttcatcctgaatggcatcaactctggcaccacctgctccaatgacctgctgcagcccaacacagaggtcttcacagatgtctgtgtggactatgacctgtatggcatcacaggccagggcagatctggcggcggaggaagcggaggaggtggcagcggtggcggtggctccggcggaggtggatccggcgtgagcaagggcgaggaggcatctggcagagccctgttccagtaccccatgaccagcaagatcgagctgaacggcgagatcaacggcaagaaattcaaggtggccggcgagggcttcacccccagcagcggcagattcaacatgcacgcctactgcaccaccggcgacctgcctatgagctgggtcgtgattgccagccccctccagtacggcttccacatgttcgcccactaccccgaggacatcacacactttttccaggaatgcttccccggcagctacaccctggaccggaccctgagaatggaaggcgacggcaccctgaccacccaccacgagtacagcctggaggacggctgcgtgacctccaagaccaccctgaatgccagcggcttcgaccctaagggcgccaccatgaccaagagcttcgtgaaacaactgcctaacgaggtgaagatcaccccccacggccccaacggcatcagactgaccagcaccgtgctgtacctgaaggaggatggcaccatccagatcggcacccaggactgcatcgtgacccctgtgggcggaaggaaagtgacccagcccaaggcccacttcctgcacacccagatcatccagaagaaggaccccaacgacacccgggaccacatcgtgcagacagaactggccgtggccggcaatctgtggcacggcatggacgagctgtacaagggtagcggtcaccaccaccaccaccactga

SEQ ID NO: 19 - protein, 525 aa, Artificial sequence
  RaTG13-RBG amino acid sequence
MARSVTLVFLVLVSLTGLYASNFRVQPTDSIVRFPNITNLCPFGEVFNATTFASVYAWNRKRISNCVADYSVLYNSTSFSTFKCYGVSPTKLNDLCFTNVYADSFVITGDEVRQIAPGQTGKIADYNYKLPDDFTGCVIAWNSKHIDAKEGGNFNYLYRLFRKANLKPFERDISTEIYQAGSKPCNGQTGLNCYYPLYRYGFYPTDGVGHQPYRVVVLSFELLNAPATVCGPKKSTNLVKNKCVNFNFNGLTGTGRSGGGGSGGGGSGGGGSGGGGSGVSKGEEASGRALFQYPMTSKIELNGEINGKKFKVAGEGFTPSSGRFNMHAYCTTGDLPMSWVVIASPLQYGFHMFAHYPEDITHFFQECFPGSYTLDRTLRMEGDGTLTTHHEYSLEDGCVTSKTTLNASGFDPKGATMTKSFVKQLPNEVKITPHGPNGIRLTSTVLYLKEDGTIQIGTQDCIVTPVGGRKVTQPKAHFLHTQIIQKKDPNDTRDHIVQTELAVAGNLWHGMDELYKGSGHHHHHH

SEQ ID NO: 20 - DNA, 1578 bp, Artificial sequence
  RaTG13-RBG nucleic acid sequence
atggcccgcagcgtgaccctggtgttcctggtgctggtgagcctgaccggtctgtacgccagcaacttccgcgtgcagcccaccgacagcatcgtgcgcttccccaacatcaccaacctgtgccccttcggcgaggtgttcaacgccaccaccttcgccagcgtgtacgcctggaaccgcaagcgcatcagcaactgcgtggccgactacagcgtgctgtacaacagcaccagcttcagcaccttcaagtgctacggcgtgagccccaccaagctgaacgacctgtgcttcaccaacgtgtacgccgacagcttcgtgatcaccggcgacgaggtgcgccagatcgcccccggccagaccggcaagatcgccgactacaactacaagctgcccgacgacttcaccggctgcgtgatcgcctggaacagcaagcacatcgacgccaaggagggcggcaacttcaactacctgtaccgcctgttccgcaaggccaacctgaagcccttcgagcgcgacatcagcaccgagatataccaggccggcagcaagccctgcaacggccagaccggcctgaactgctactaccccctgtaccgctacggcttctaccccaccgacggcgtgggccaccagccctaccgcgtggtggtgctgagcttcgagctgctgaacgcccccgccaccgtgtgcggccccaagaagagcaccaacctggtgaagaacaagtgcgtgaacttcaacttcaacggcctgaccggcaccggcagatctggcggcggaggaagcggaggaggtggcagcggtggcggtggctccggcggaggtggatccggcgtgagcaagggcgaggaggcatctggcagagccctgttccagtaccccatgaccagcaagatcgagctgaacggcgagatcaacggcaagaaattcaaggtggccggcgagggcttcacccccagcagcggcagattcaacatgcacgcctactgcaccaccggcgacctgcctatgagctgggtcgtgattgccagccccctccagtacggcttccacatgttcgcccactaccccgaggacatcacacactttttccaggaatgcttccccggcagctacaccctggaccggaccctgagaatggaaggcgacggcaccctgaccacccaccacgagtacagcctggaggacggctgcgtgacctccaagaccaccctgaatgccagcggcttcgaccctaagggcgccaccatgaccaagagcttcgtgaaacaactgcctaacgaggtgaagatcaccccccacggccccaacggcatcagactgaccagcaccgtgctgtacctgaaggaggatggcaccatccagatcggcacccaggactgcatcgtgacccctgtgggcggaaggaaagtgacccagcccaaggcccacttcctgcacacccagatcatccagaagaaggaccccaacgacacccgggaccacatcgtgcagacagaactggccgtggccggcaatctgtggcacggcatggacgagctgtacaagggtagcggtcaccaccaccaccaccactga

SEQ ID NO: 21 - protein, 1192 aa, Artificial sequence
  SARS-CoV2-Secd amino acid sequence
VNLTTRTQLPPAYTNSFTRGVYYPDKVFRSSVLHSTQDLFLPFFSNVTWFHAIHVSGTNGTKRFDNPVLPFNDGVYFASTEKSNIIRGWIFGTTLDSKTQSLLIVNNATNVVIKVCEFQFCNDPFLGVYYHKNNKSWMESEFRVYSSANNCTFEYVSQPFLMDLEGKQGNFKNLREFVFKNIDGYFKIYSKHTPINLVRDLPQGFSALEPLVDLPIGINITRFQTLLALHRSYLTPGDSSSGWTAGAAAYYVGYLQPRTFLLKYNENGTITDAVDCALDPLSETKCTLKSFTVEKGIYQTSNFRVQPTESIVRFPNITNLCPFGEVFNATRFASVYAWNRKRISNCVADYSVLYNSASFSTFKCYGVSPTKLNDLCFTNVYADSFVIRGDEVRQIAPGQTGKIADYNYKLPDDFTGCVIAWNSNNLDSKVGGNYNYLYRLFRKSNLKPFERDISTEIYQAGSTPCNGVEGFNCYFPLQSYGFQPTNGVGYQPYRVVVLSFELLHAPATVCGPKKSTNLVKNKCVNFNFNGLTGTGVLTESNKKFLPFQQFGRDIADTTDAVRDPQTLEILDITPCSFGGVSVITPGTNTSNQVAVLYQDVNCTEVPVAIHADQLTPTWRVYSTGSNVFQTRAGCLIGAEHVNNSYECDIPIGAGICASYQTQTNSPGSASSVASQSIIAYTMSLGAENSVAYSNNSIAIPTNFTISVTTEILPVSMTKTSVDCTMYICGDSTECSNLLLQYGSFCTQLNRALTGIAVEQDKNTQEVFAQVKQIYKTPPIKDFGGFNFSQILPDPSKPSKRSFIEDLLFNKVTLADAGFIKQYGDCLGDIAARDLICAQKFNGLTVLPPLLTDEMIAQYTSALLAGTITSGWTFGAGAALQIPFAMQMAYRFNGIGVTQNVLYENQKLIANQFNSAIGKIQDSLSSTASALGKLQDVVNQNAQALNTLVKQLSSNFGAISSVLNDILSRLDKVEAEVQIDRLITGRLQSLQTYVTQQLIRAAEIRASANLAATKMSECVLGQSKRVDFCGKGYHLMSFPQSAPHGVVFLHVTYVPAQEKNFTTAPAICHDGKAHFPREGVFVSNGTHWFVTQRNFYEPQIITTDNTFVSGNCDVVIGIVNNTVYDPLQPELDSFKEELDKYFKNHTSPDVDLGDISGINASVVNIQKEIDRLNEVAKNLNESLIDLQELGKYE

SEQ ID NO: 22 - DNA, 3576 bp, Artificial sequence
  SARS-CoV2-Secd nucleotide sequence
gtgaacctgaccacccgcacccagctgccccccgcctacaccaacagcttcacccgcggcgtgtactaccccgacaaggtgttccgcagcagcgtgctgcacagcacccaggacctgttcctgcccttcttcagcaacgtgacctggttccacgccatccacgtgagcggcaccaacggcaccaagcgcttcgacaaccccgtgctgcccttcaacgacggcgtgtacttcgccagcaccgagaagagcaacatcatccgcggctggatcttcggcaccaccctggacagcaagacccagagcctgctgatcgtgaacaacgccaccaacgtggtgatcaaggtgtgcgagttccagttctgcaacgaccccttcctgggcgtgtactaccacaagaacaacaagagctggatggagagcgagttccgcgtgtacagcagcgccaacaactgcaccttcgagtacgtgagccagcccttcctgatggacctggagggcaagcagggcaacttcaagaacctgcgcgagttcgtgttcaagaacatcgacggctacttcaagatatacagcaagcacacccccatcaacctggtgcgcgacctgccccagggcttcagcgccctggagcccctggtggacctgcccatcggcatcaacatcacccgcttccagaccctgctggccctgcaccgcagctacctgacccccggcgacagcagcagcggctggaccgccggcgccgccgcctactacgtgggctacctgcagccccgcaccttcctgctgaagtacaacgagaacggcaccatcaccgacgccgtggactgcgccctggaccccctgagcgagaccaagtgcaccctgaagagcttcaccgtggagaagggcatctaccagaccagcaacttccgcgtgcagcccaccgagagcatcgtgcgcttccccaacatcaccaacctgtgccccttcggcgaggtgttcaacgccacccgcttcgccagcgtgtacgcctggaaccgcaagcgcatcagcaactgcgtggccgactacagcgtgctgtacaacagcgccagcttcagcaccttcaagtgctacggcgtgagccccaccaagctgaacgacctgtgcttcaccaacgtgtacgccgacagcttcgtgatccgcggcgacgaggtgcgccagatcgcccccggccagaccggcaagatcgccgactacaactacaagctgcccgacgacttcaccggctgcgtgatcgcctggaacagcaacaacctggacagcaaggtgggcggcaactacaactacctgtaccgcctgttccgcaagagcaacctgaagcccttcgagcgcgacatcagcaccgagatataccaggccggcagcaccccctgcaacggcgtggagggcttcaactgctacttccccctgcagagctacggcttccagcccaccaacggcgtgggctaccagccctaccgcgtggtggtgctgagcttcgagctgctgcacgcccccgccaccgtgtgcggccccaagaagagcaccaacctggtgaagaacaagtgcgtgaacttcaacttcaacggcctgaccggcaccggcgtgctgaccgagagcaacaagaagttcctgcccttccagcagttcggccgcgacatcgccgacaccaccgacgccgtgcgcgacccccagaccctggagatcctggacatcaccccctgcagcttcggcggcgtgagcgtgatcacccccggcaccaacaccagcaaccaggtggccgtgctgtaccaggacgtgaactgcaccgaggtgcccgtggccatccacgccgaccagctgacccccacctggcgcgtgtacagcaccggcagcaacgtgttccagacccgcgccggctgcctgatcggcgccgagcacgtgaacaacagctacgagtgcgacatccccatcggcgccggcatctgcgccagctaccagacccagaccaacagccccggtagcgcgagctctgtggccagccagagcatcatcgcctacaccatgagcctgggcgccgagaacagcgtggcctacagcaacaacagcatcgccatccccaccaacttcaccatcagcgtgaccaccgagatcctgcccgtgagcatgaccaagaccagcgtggactgcaccatgtacatctgcggcgacagcaccgagtgcagcaacctgctgctgcagtacggcagcttctgcacccagctgaaccgcgccctgaccggcatcgccgtggagcaggacaagaacacccaggaggtgttcgcccaggtgaagcagatatacaagaccccccccatcaaggacttcggcggcttcaacttcagccagatcctgcccgaccccagcaagcccagcaagcgcagcttcatcgaggacctgctgttcaacaaggtgaccctggccgacgccggcttcatcaagcagtacggcgactgcctgggcgacatcgccgcccgcgacctgatctgcgcccagaagttcaacggcctgaccgtgctgccccccctgctgaccgacgagatgatcgcccagtacaccagcgccctgctggccggcaccatcaccagcggctggaccttcggcgccggcgccgccctgcagatccccttcgccatgcagatggcctaccgcttcaacggcatcggcgtgacccagaacgtgctgtacgagaaccagaagctgatcgccaaccagttcaacagcgccatcggcaagatccaggacagcctgagcagcaccgccagcgccctgggcaagctgcaggacgtggtgaaccagaacgcccaggccctgaacaccctggtgaagcagctgagcagcaacttcggcgccatcagcagcgtgctgaacgacatcctgagccgcctggacaaggtggaggccgaggtgcagatcgaccgcctgatcaccggccgcctgcagagcctgcagacctacgtgacccagcagctgatccgcgccgccgagatccgcgccagcgccaacctggccgccaccaagatgagcgagtgcgtgctgggccagagcaagcgcgtggacttctgcggcaagggctaccacctgatgagcttcccccagagcgccccccacggcgtggtgttcctgcacgtgacctacgtgcccgcccaggagaagaacttcaccaccgcccccgccatctgccacgacggcaaggcccacttcccccgcgagggcgtgttcgtgagcaacggcacccactggttcgtgacccagcgcaacttctacgagccccagatcatcaccaccgacaacaccttcgtgagcggcaactgcgacgtggtgatcggcatcgtgaacaacaccgtgtacgaccccctgcagcccgagctggacagcttcaaggaggagctggacaagtacttcaagaaccacaccagccccgacgtggacctgggcgacatcagcggcatcaacgctagcgtggtgaacatccagaaggagatcgaccgcctgaacgaggtggccaagaacctgaacgagagcctgatcgacctgcaggagctgggcaagtacgag

SEQ ID NO: 23 - DNA, 81 bp, Artificial sequence
  TFD nucleotide sequence
tacatccccgaggccccccgcgacggccaggcctacgtgcgcaaggacggcgagtgggtgctgctgagcaccttcctgggc

SEQ ID NO: 24 - DNA, 4542 bp, Artificial sequence
  SARS-CoV2-STG nucleotide sequence
atggcccgcagcgtgaccctggtgttcctggtgctggtgagcctgaccggtctgtacgccgtgaacctgaccacccgcacccagctgccccccgcctacaccaacagcttcacccgcggcgtgtactaccccgacaaggtgttccgcagcagcgtgctgcacagcacccaggacctgttcctgcccttcttcagcaacgtgacctggttccacgccatccacgtgagcggcaccaacggcaccaagcgcttcgacaaccccgtgctgcccttcaacgacggcgtgtacttcgccagcaccgagaagagcaacatcatccgcggctggatcttcggcaccaccctggacagcaagacccagagcctgctgatcgtgaacaacgccaccaacgtggtgatcaaggtgtgcgagttccagttctgcaacgaccccttcctgggcgtgtactaccacaagaacaacaagagctggatggagagcgagttccgcgtgtacagcagcgccaacaactgcaccttcgagtacgtgagccagcccttcctgatggacctggagggcaagcagggcaacttcaagaacctgcgcgagttcgtgttcaagaacatcgacggctacttcaagatatacagcaagcacacccccatcaacctggtgcgcgacctgccccagggcttcagcgccctggagcccctggtggacctgcccatcggcatcaacatcacccgcttccagaccctgctggccctgcaccgcagctacctgacccccggcgacagcagcagcggctggaccgccggcgccgccgcctactacgtgggctacctgcagccccgcaccttcctgctgaagtacaacgagaacggcaccatcaccgacgccgtggactgcgccctggaccccctgagcgagaccaagtgcaccctgaagagcttcaccgtggagaagggcatctaccagaccagcaacttccgcgtgcagcccaccgagagcatcgtgcgcttccccaacatcaccaacctgtgccccttcggcgaggtgttcaacgccacccgcttcgccagcgtgtacgcctggaaccgcaagcgcatcagcaactgcgtggccgactacagcgtgctgtacaacagcgccagcttcagcaccttcaagtgctacggcgtgagccccaccaagctgaacgacctgtgcttcaccaacgtgtacgccgacagcttcgtgatccgcggcgacgaggtgcgccagatcgcccccggccagaccggcaagatcgccgactacaactacaagctgcccgacgacttcaccggctgcgtgatcgcctggaacagcaacaacctggacagcaaggtgggcggcaactacaactacctgtaccgcctgttccgcaagagcaacctgaagcccttcgagcgcgacatcagcaccgagatataccaggccggcagcaccccctgcaacggcgtggagggcttcaactgctacttccccctgcagagctacggcttccagcccaccaacggcgtgggctaccagccctaccgcgtggtggtgctgagcttcgagctgctgcacgcccccgccaccgtgtgcggccccaagaagagcaccaacctggtgaagaacaagtgcgtgaacttcaacttcaacggcctgaccggcaccggcgtgctgaccgagagcaacaagaagttcctgcccttccagcagttcggccgcgacatcgccgacaccaccgacgccgtgcgcgacccccagaccctggagatcctggacatcaccccctgcagcttcggcggcgtgagcgtgatcacccccggcaccaacaccagcaaccaggtggccgtgctgtaccaggacgtgaactgcaccgaggtgcccgtggccatccacgccgaccagctgacccccacctggcgcgtgtacagcaccggcagcaacgtgttccagacccgcgccggctgcctgatcggcgccgagcacgtgaacaacagctacgagtgcgacatccccatcggcgccggcatctgcgccagctaccagacccagaccaacagccccggtagcgcgagctctgtggccagccagagcatcatcgcctacaccatgagcctgggcgccgagaacagcgtggcctacagcaacaacagcatcgccatccccaccaacttcaccatcagcgtgaccaccgagatcctgcccgtgagcatgaccaagaccagcgtggactgcaccatgtacatctgcggcgacagcaccgagtgcagcaacctgctgctgcagtacggcagcttctgcacccagctgaaccgcgccctgaccggcatcgccgtggagcaggacaagaacacccaggaggtgttcgcccaggtgaagcagatatacaagaccccccccatcaaggacttcggcggcttcaacttcagccagatcctgcccgaccccagcaagcccagcaagcgcagcttcatcgaggacctgctgttcaacaaggtgaccctggccgacgccggcttcatcaagcagtacggcgactgcctgggcgacatcgccgcccgcgacctgatctgcgcccagaagttcaacggcctgaccgtgctgccccccctgctgaccgacgagatgatcgcccagtacaccagcgccctgctggccggcaccatcaccagcggctggaccttcggcgccggcgccgccctgcagatccccttcgccatgcagatggcctaccgcttcaacggcatcggcgtgacccagaacgtgctgtacgagaaccagaagctgatcgccaaccagttcaacagcgccatcggcaagatccaggacagcctgagcagcaccgccagcgccctgggcaagctgcaggacgtggtgaaccagaacgcccaggccctgaacaccctggtgaagcagctgagcagcaacttcggcgccatcagcagcgtgctgaacgacatcctgagccgcctggacaaggtggaggccgaggtgcagatcgaccgcctgatcaccggccgcctgcagagcctgcagacctacgtgacccagcagctgatccgcgccgccgagatccgcgccagcgccaacctggccgccaccaagatgagcgagtgcgtgctgggccagagcaagcgcgtggacttctgcggcaagggctaccacctgatgagcttcccccagagcgccccccacggcgtggtgttcctgcacgtgacctacgtgcccgcccaggagaagaacttcaccaccgcccccgccatctgccacgacggcaaggcccacttcccccgcgagggcgtgttcgtgagcaacggcacccactggttcgtgacccagcgcaacttctacgagccccagatcatcaccaccgacaacaccttcgtgagcggcaactgcgacgtggtgatcggcatcgtgaacaacaccgtgtacgaccccctgcagcccgagctggacagcttcaaggaggagctggacaagtacttcaagaaccacaccagccccgacgtggacctgggcgacatcagcggcatcaacgctagcgtggtgaacatccagaaggagatcgaccgcctgaacgaggtggccaagaacctgaacgagagcctgatcgacctgcaggagctgggcaagtacgaattcggttacatccccgaggccccccgcgacggccaggcctacgtgcgcaaggacggcgagtgggtgctgctgagcaccttcctgggcgtcgacggcggcggaggaagcggaggaggtggcagcggtggcggtggctccggcggaggtggatccggcgtgagcaagggcgaggaggcatctggcagagccctgttccagtaccccatgaccagcaagatcgagctgaacggcgagatcaacggcaagaaattcaaggtggccggcgagggcttcacccccagcagcggcagattcaacatgcacgcctactgcaccaccggcgacctgcctatgagctgggtcgtgattgccagccccctccagtacggcttccacatgttcgcccactaccccgaggacatcacacactttttccaggaatgcttccccggcagctacaccctggaccggaccctgagaatggaaggcgacggcaccctgaccacccaccacgagtacagcctggaggacggctgcgtgacctccaagaccaccctgaatgccagcggcttcgaccctaagggcgccaccatgaccaagagcttcgtgaaacaactgcctaacgaggtgaagatcaccccccacggccccaacggcatcagactgaccagcaccgtgctgtacctgaaggaggatggcaccatccagatcggcacccaggactgcatcgtgacccctgtgggcggaaggaaagtgacccagcccaaggcccacttcctgcacacccagatcatccagaagaaggaccccaacgacacccgggaccacatcgtgcagacagaactggccgtggccggcaatctgtggcacggcatggacgagctgtacaagagcctcgagcatcaccaccaccaccaccaccactaa

SEQ ID NO: 25 - DNA, 4533 bp, Artificial sequence
  SARS-CoV2-STN nucleotide sequence
atggcccgcagcgtgaccctggtgttcctggtgctggtgagcctgaccggtctgtacgccgtgaacctgaccacccgcacccagctgccccccgcctacaccaacagcttcacccgcggcgtgtactaccccgacaaggtgttccgcagcagcgtgctgcacagcacccaggacctgttcctgcccttcttcagcaacgtgacctggttccacgccatccacgtgagcggcaccaacggcaccaagcgcttcgacaaccccgtgctgcccttcaacgacggcgtgtacttcgccagcaccgagaagagcaacatcatccgcggctggatcttcggcaccaccctggacagcaagacccagagcctgctgatcgtgaacaacgccaccaacgtggtgatcaaggtgtgcgagttccagttctgcaacgaccccttcctgggcgtgtactaccacaagaacaacaagagctggatggagagcgagttccgcgtgtacagcagcgccaacaactgcaccttcgagtacgtgagccagcccttcctgatggacctggagggcaagcagggcaacttcaagaacctgcgcgagttcgtgttcaagaacatcgacggctacttcaagatatacagcaagcacacccccatcaacctggtgcgcgacctgccccagggcttcagcgccctggagcccctggtggacctgcccatcggcatcaacatcacccgcttccagaccctgctggccctgcaccgcagctacctgacccccggcgacagcagcagcggctggaccgccggcgccgccgcctactacgtgggctacctgcagccccgcaccttcctgctgaagtacaacgagaacggcaccatcaccgacgccgtggactgcgccctggaccccctgagcgagaccaagtgcaccctgaagagcttcaccgtggagaagggcatctaccagaccagcaacttccgcgtgcagcccaccgagagcatcgtgcgcttccccaacatcaccaacctgtgccccttcggcgaggtgttcaacgccacccgcttcgccagcgtgtacgcctggaaccgcaagcgcatcagcaactgcgtggccgactacagcgtgctgtacaacagcgccagcttcagcaccttcaagtgctacggcgtgagccccaccaagctgaacgacctgtgcttcaccaacgtgtacgccgacagcttcgtgatccgcggcgacgaggtgcgccagatcgcccccggccagaccggcaagatcgccgactacaactacaagctgcccgacgacttcaccggctgcgtgatcgcctggaacagcaacaacctggacagcaaggtgggcggcaactacaactacctgtaccgcctgttccgcaagagcaacctgaagcccttcgagcgcgacatcagcaccgagatataccaggccggcagcaccccctgcaacggcgtggagggcttcaactgctacttccccctgcagagctacggcttccagcccaccaacggcgtgggctaccagccctaccgcgtggtggtgctgagcttcgagctgctgcacgcccccgccaccgtgtgcggccccaagaagagcaccaacctggtgaagaacaagtgcgtgaacttcaacttcaacggcctgaccggcaccggcgtgctgaccgagagcaacaagaagttcctgcccttccagcagttcggccgcgacatcgccgacaccaccgacgccgtgcgcgacccccagaccctggagatcctggacatcaccccctgcagcttcggcggcgtgagcgtgatcacccccggcaccaacaccagcaaccaggtggccgtgctgtaccaggacgtgaactgcaccgaggtgcccgtggccatccacgccgaccagctgacccccacctggcgcgtgtacagcaccggcagcaacgtgttccagacccgcgccggctgcctgatcggcgccgagcacgtgaacaacagctacgagtgcgacatccccatcggcgccggcatctgcgccagctaccagacccagaccaacagccccggtagcgcgagctctgtggccagccagagcatcatcgcctacaccatgagcctgggcgccgagaacagcgtggcctacagcaacaacagcatcgccatccccaccaacttcaccatcagcgtgaccaccgagatcctgcccgtgagcatgaccaagaccagcgtggactgcaccatgtacatctgcggcgacagcaccgagtgcagcaacctgctgctgcagtacggcagcttctgcacccagctgaaccgcgccctgaccggcatcgccgtggagcaggacaagaacacccaggaggtgttcgcccaggtgaagcagatatacaagaccccccccatcaaggacttcggcggcttcaacttcagccagatcctgcccgaccccagcaagcccagcaagcgcagcttcatcgaggacctgctgttcaacaaggtgaccctggccgacgccggcttcatcaagcagtacggcgactgcctgggcgacatcgccgcccgcgacctgatctgcgcccagaagttcaacggcctgaccgtgctgccccccctgctgaccgacgagatgatcgcccagtacaccagcgccctgctggccggcaccatcaccagcggctggaccttcggcgccggcgccgccctgcagatccccttcgccatgcagatggcctaccgcttcaacggcatcggcgtgacccagaacgtgctgtacgagaaccagaagctgatcgccaaccagttcaacagcgccatcggcaagatccaggacagcctgagcagcaccgccagcgccctgggcaagctgcaggacgtggtgaaccagaacgcccaggccctgaacaccctggtgaagcagctgagcagcaacttcggcgccatcagcagcgtgctgaacgacatcctgagccgcctggacaaggtggaggccgaggtgcagatcgaccgcctgatcaccggccgcctgcagagcctgcagacctacgtgacccagcagctgatccgcgccgccgagatccgcgccagcgccaacctggccgccaccaagatgagcgagtgcgtgctgggccagagcaagcgcgtggacttctgcggcaagggctaccacctgatgagcttcccccagagcgccccccacggcgtggtgttcctgcacgtgacctacgtgcccgcccaggagaagaacttcaccaccgcccccgccatctgccacgacggcaaggcccacttcccccgcgagggcgtgttcgtgagcaacggcacccactggttcgtgacccagcgcaacttctacgagccccagatcatcaccaccgacaacaccttcgtgagcggcaactgcgacgtggtgatcggcatcgtgaacaacaccgtgtacgaccccctgcagcccgagctggacagcttcaaggaggagctggacaagtacttcaagaaccacaccagccccgacgtggacctgggcgacatcagcggcatcaacgctagcgtggtgaacatccagaaggagatcgaccgcctgaacgaggtggccaagaacctgaacgagagcctgatcgacctgcaggagctgggcaagtacgaattcggttacatccccgaggccccccgcgacggccaggcctacgtgcgcaaggacggcgagtgggtgctgctgagcaccttcctgggcgtcgacggcggcggaggaagcggaggaggtggcagcggtggcggtggctccggcggaggtggatccggcgtgagcaagggcgaggaggacaacatggccagcctgcccgccacccacgagctgcacatcttcggcagcatcaacggcgtggacttcgacatggtgggccagggcaccggcaaccccaacgacggctacgaggagctgaacctgaagagcaccaagggcgacctgcagttcagcccctggatcttagtgccccacatcggctacggcttccaccagtacctgccctaccccgacggcatgagccccttccaggccgccatggtggacggcagcggctaccaggtgcaccgcaccatgcagttcgaggacggcgccagcctgaccgtgaactaccgctacacctacgagggcagccacatcaagggcgaggcccaggtgaagggcaccggcttccccgccgacggccccgtgatgaccaacagcctgaccgccgccgactggtgccgcagcaagaagacctaccccaacgacaagaccatcatcagcaccttcaagtggagctacaccaccggcaacggcaagcgctaccgcagcaccgcccgcaccacctacaccttcgccaagcccatggccgccaactacctgaagaaccagcccatgtacgtgttccgcaagaccgagctgaagcacagcaagaccgagctgaacttcaaggagtggcagaaggccttcaccgacgtgatgggcatggacgagctgtacaagagcctcgagcatcaccaccaccaccaccaccactaa

SEQ ID NO: 26 - protein, 1513 aa, Artificial sequence
  SARS-CoV2-STG amino acid sequence
MARSVTLVFLVLVSLTGLYAVNLTTRTQLPPAYTNSFTRGVYYPDKVFRSSVLHSTQDLFLPFFSNVTWFHAIHVSGTNGTKRFDNPVLPFNDGVYFASTEKSNIIRGWIFGTTLDSKTQSLLIVNNATNVVIKVCEFQFCNDPFLGVYYHKNNKSWMESEFRVYSSANNCTFEYVSQPFLMDLEGKQGNFKNLREFVFKNIDGYFKIYSKHTPINLVRDLPQGFSALEPLVDLPIGINITRFQTLLALHRSYLTPGDSSSGWTAGAAAYYVGYLQPRTFLLKYNENGTITDAVDCALDPLSETKCTLKSFTVEKGIYQTSNFRVQPTESIVRFPNITNLCPFGEVFNATRFASVYAWNRKRISNCVADYSVLYNSASFSTFKCYGVSPTKLNDLCFTNVYADSFVIRGDEVRQIAPGQTGKIADYNYKLPDDFTGCVIAWNSNNLDSKVGGNYNYLYRLFRKSNLKPFERDISTEIYQAGSTPCNGVEGFNCYFPLQSYGFQPTNGVGYQPYRVVVLSFELLHAPATVCGPKKSTNLVKNKCVNFNFNGLTGTGVLTESNKKFLPFQQFGRDIADTTDAVRDPQTLEILDITPCSFGGVSVITPGTNTSNQVAVLYQDVNCTEVPVAIHADQLTPTWRVYSTGSNVFQTRAGCLIGAEHVNNSYECDIPIGAGICASYQTQTNSPGSASSVASQSIIAYTMSLGAENSVAYSNNSIAIPTNFTISVTTEILPVSMTKTSVDCTMYICGDSTECSNLLLQYGSFCTQLNRALTGIAVEQDKNTQEVFAQVKQIYKTPPIKDFGGFNFSQILPDPSKPSKRSFIEDLLFNKVTLADAGFIKQYGDCLGDIAARDLICAQKFNGLTVLPPLLTDEMIAQYTSALLAGTITSGWTFGAGAALQIPFAMQMAYRFNGIGVTQNVLYENQKLIANQFNSAIGKIQDSLSSTASALGKLQDVVNQNAQALNTLVKQLSSNFGAISSVLNDILSRLDKVEAEVQIDRLITGRLQSLQTYVTQQLIRAAEIRASANLAATKMSECVLGQSKRVDFCGKGYHLMSFPQSAPHGVVFLHVTYVPAQEKNFTTAPAICHDGKAHFPREGVFVSNGTHWFVTQRNFYEPQIITTDNTFVSGNCDVVIGIVNNTVYDPLQPELDSFKEELDKYFKNHTSPDVDLGDISGINASVVNIQKEIDRLNEVAKNLNESLIDLQELGKYEFGYIPEAPRDGQAYVRKDGEWVLLSTFLGVDGGGGSGGGGSGGGGSGGGGSGVSKGEEASGRALFQYPMTSKIELNGEINGKKFKVAGEGFTPSSGRFNMHAYCTTGDLPMSWVVIASPLQYGFHMFAHYPEDITHFFQECFPGSYTLDRTLRMEGDGTLTTHHEYSLEDGCVTSKTTLNASGFDPKGATMTKSFVKQLPNEVKITPHGPNGIRLTSTVLYLKEDGTIQIGTQDCIVTPVGGRKVTQPKAHFLHTQIIQKKDPNDTRDHIVQTELAVAGNLWHGMDELYKSLEHHHHHHHH

SEQ ID NO: 27 - protein, 1510 aa, Artificial sequence
  SARS-CoV2-STN amino acid sequence
MARSVTLVFLVLVSLTGLYAVNLTTRTQLPPAYTNSFTRGVYYPDKVFRSSVLHSTQDLFLPFFSNVTWFHAIHVSGTNGTKRFDNPVLPFNDGVYFASTEKSNIIRGWIFGTTLDSKTQSLLIVNNATNVVIKVCEFQFCNDPFLGVYYHKNNKSWMESEFRVYSSANNCTFEYVSQPFLMDLEGKQGNFKNLREFVFKNIDGYFKIYSKHTPINLVRDLPQGFSALEPLVDLPIGINITRFQTLLALHRSYLTPGDSSSGWTAGAAAYYVGYLQPRTFLLKYNENGTITDAVDCALDPLSETKCTLKSFTVEKGIYQTSNFRVQPTESIVRFPNITNLCPFGEVFNATRFASVYAWNRKRISNCVADYSVLYNSASFSTFKCYGVSPTKLNDLCFTNVYADSFVIRGDEVRQIAPGQTGKIADYNYKLPDDFTGCVIAWNSNNLDSKVGGNYNYLYRLFRKSNLKPFERDISTEIYQAGSTPCNGVEGFNCYFPLQSYGFQPTNGVGYQPYRVVVLSFELLHAPATVCGPKKSTNLVKNKCVNFNFNGLTGTGVLTESNKKFLPFQQFGRDIADTTDAVRDPQTLEILDITPCSFGGVSVITPGTNTSNQVAVLYQDVNCTEVPVAIHADQLTPTWRVYSTGSNVFQTRAGCLIGAEHVNNSYECDIPIGAGICASYQTQTNSPGSASSVASQSIIAYTMSLGAENSVAYSNNSIAIPTNFTISVTTEILPVSMTKTSVDCTMYICGDSTECSNLLLQYGSFCTQLNRALTGIAVEQDKNTQEVFAQVKQIYKTPPIKDFGGFNFSQILPDPSKPSKRSFIEDLLFNKVTLADAGFIKQYGDCLGDIAARDLICAQKFNGLTVLPPLLTDEMIAQYTSALLAGTITSGWTFGAGAALQIPFAMQMAYRFNGIGVTQNVLYENQKLIANQFNSAIGKIQDSLSSTASALGKLQDVVNQNAQALNTLVKQLSSNFGAISSVLNDILSRLDKVEAEVQIDRLITGRLQSLQTYVTQQLIRAAEIRASANLAATKMSECVLGQSKRVDFCGKGYHLMSFPQSAPHGVVFLHVTYVPAQEKNFTTAPAICHDGKAHFPREGVFVSNGTHWFVTQRNFYEPQIITTDNTFVSGNCDVVIGIVNNTVYDPLQPELDSFKEELDKYFKNHTSPDVDLGDISGINASVVNIQKEIDRLNEVAKNLNESLIDLQELGKYEFGYIPEAPRDGQAYVRKDGEWVLLSTFLGVDGGGGSGGGGSGGGGSGGGGSGVSKGEEDNMASLPATHELHIFGSINGVDFDMVGQGTGNPNDGYEELNLKSTKGDLQFSPWILVPHIGYGFHQYLPYPDGMSPFQAAMVDGSGYQVHRTMQFEDGASLTVNYRYTYEGSHIKGEAQVKGTGFPADGPVMTNSLTAADWCRSKKTYPNDKTIISTFKWSYTTGNGKRYRSTARTTYTFAKPMAANYLKNQPMYVFRKTELKHSKTELNFKEWQKAFTDVMGMDELYKSLEHHHHHHHH

SEQ ID NO: 28 - DNA, 3765 bp, Artificial sequence
  SARS-CoV2-ST nucleic acid sequence
atggcccgcagcgtgaccctggtgttcctggtgctggtgagcctgaccggtctgtacgccgtgaacctgaccacccgcacccagctgccccccgcctacaccaacagcttcacccgcggcgtgtactaccccgacaaggtgttccgcagcagcgtgctgcacagcacccaggacctgttcctgcccttcttcagcaacgtgacctggttccacgccatccacgtgagcggcaccaacggcaccaagcgcttcgacaaccccgtgctgcccttcaacgacggcgtgtacttcgccagcaccgagaagagcaacatcatccgcggctggatcttcggcaccaccctggacagcaagacccagagcctgctgatcgtgaacaacgccaccaacgtggtgatcaaggtgtgcgagttccagttctgcaacgaccccttcctgggcgtgtactaccacaagaacaacaagagctggatggagagcgagttccgcgtgtacagcagcgccaacaactgcaccttcgagtacgtgagccagcccttcctgatggacctggagggcaagcagggcaacttcaagaacctgcgcgagttcgtgttcaagaacatcgacggctacttcaagatatacagcaagcacacccccatcaacctggtgcgcgacctgccccagggcttcagcgccctggagcccctggtggacctgcccatcggcatcaacatcacccgcttccagaccctgctggccctgcaccgcagctacctgacccccggcgacagcagcagcggctggaccgccggcgccgccgcctactacgtgggctacctgcagccccgcaccttcctgctgaagtacaacgagaacggcaccatcaccgacgccgtggactgcgccctggaccccctgagcgagaccaagtgcaccctgaagagcttcaccgtggagaagggcatctaccagaccagcaacttccgcgtgcagcccaccgagagcatcgtgcgcttccccaacatcaccaacctgtgccccttcggcgaggtgttcaacgccacccgcttcgccagcgtgtacgcctggaaccgcaagcgcatcagcaactgcgtggccgactacagcgtgctgtacaacagcgccagcttcagcaccttcaagtgctacggcgtgagccccaccaagctgaacgacctgtgcttcaccaacgtgtacgccgacagcttcgtgatccgcggcgacgaggtgcgccagatcgcccccggccagaccggcaagatcgccgactacaactacaagctgcccgacgacttcaccggctgcgtgatcgcctggaacagcaacaacctggacagcaaggtgggcggcaactacaactacctgtaccgcctgttccgcaagagcaacctgaagcccttcgagcgcgacatcagcaccgagatataccaggccggcagcaccccctgcaacggcgtggagggcttcaactgctacttccccctgcagagctacggcttccagcccaccaacggcgtgggctaccagccctaccgcgtggtggtgctgagcttcgagctgctgcacgcccccgccaccgtgtgcggccccaagaagagcaccaacctggtgaagaacaagtgcgtgaacttcaacttcaacggcctgaccggcaccggcgtgctgaccgagagcaacaagaagttcctgcccttccagcagttcggccgcgacatcgccgacaccaccgacgccgtgcgcgacccccagaccctggagatcctggacatcaccccctgcagcttcggcggcgtgagcgtgatcacccccggcaccaacaccagcaaccaggtggccgtgctgtaccaggacgtgaactgcaccgaggtgcccgtggccatccacgccgaccagctgacccccacctggcgcgtgtacagcaccggcagcaacgtgttccagacccgcgccggctgcctgatcggcgccgagcacgtgaacaacagctacgagtgcgacatccccatcggcgccggcatctgcgccagctaccagacccagaccaacagccccggtagcgcgagctctgtggccagccagagcatcatcgcctacaccatgagcctgggcgccgagaacagcgtggcctacagcaacaacagcatcgccatccccaccaacttcaccatcagcgtgaccaccgagatcctgcccgtgagcatgaccaagaccagcgtggactgcaccatgtacatctgcggcgacagcaccgagtgcagcaacctgctgctgcagtacggcagcttctgcacccagctgaaccgcgccctgaccggcatcgccgtggagcaggacaagaacacccaggaggtgttcgcccaggtgaagcagatatacaagaccccccccatcaaggacttcggcggcttcaacttcagccagatcctgcccgaccccagcaagcccagcaagcgcagcttcatcgaggacctgctgttcaacaaggtgaccctggccgacgccggcttcatcaagcagtacggcgactgcctgggcgacatcgccgcccgcgacctgatctgcgcccagaagttcaacggcctgaccgtgctgccccccctgctgaccgacgagatgatcgcccagtacaccagcgccctgctggccggcaccatcaccagcggctggaccttcggcgccggcgccgccctgcagatccccttcgccatgcagatggcctaccgcttcaacggcatcggcgtgacccagaacgtgctgtacgagaaccagaagctgatcgccaaccagttcaacagcgccatcggcaagatccaggacagcctgagcagcaccgccagcgccctgggcaagctgcaggacgtggtgaaccagaacgcccaggccctgaacaccctggtgaagcagctgagcagcaacttcggcgccatcagcagcgtgctgaacgacatcctgagccgcctggacaaggtggaggccgaggtgcagatcgaccgcctgatcaccggccgcctgcagagcctgcagacctacgtgacccagcagctgatccgcgccgccgagatccgcgccagcgccaacctggccgccaccaagatgagcgagtgcgtgctgggccagagcaagcgcgtggacttctgcggcaagggctaccacctgatgagcttcccccagagcgccccccacggcgtggtgttcctgcacgtgacctacgtgcccgcccaggagaagaacttcaccaccgcccccgccatctgccacgacggcaaggcccacttcccccgcgagggcgtgttcgtgagcaacggcacccactggttcgtgacccagcgcaacttctacgagccccagatcatcaccaccgacaacaccttcgtgagcggcaactgcgacgtggtgatcggcatcgtgaacaacaccgtgtacgaccccctgcagcccgagctggacagcttcaaggaggagctggacaagtacttcaagaaccacaccagccccgacgtggacctgggcgacatcagcggcatcaacgctagcgtggtgaacatccagaaggagatcgaccgcctgaacgaggtggccaagaacctgaacgagagcctgatcgacctgcaggagctgggcaagtacgagcagggatccggttacatccccgaggccccccgcgacggccaggcctacgtgcgcaaggacggcgagtgggtgctgctgagcaccttcctgggcagcctcgagcatcaccaccaccaccaccaccactaa

SEQ ID NO: 29 - protein, 1254 aa, Artificial sequence
  SARS-CoV2-ST amino acid sequence
MARSVTLVFLVLVSLTGLYAVNLTTRTQLPPAYTNSFTRGVYYPDKVFRSSVLHSTQDLFLPFFSNVTWFHAIHVSGTNGTKRFDNPVLPFNDGVYFASTEKSNIIRGWIFGTTLDSKTQSLLIVNNATNVVIKVCEFQFCNDPFLGVYYHKNNKSWMESEFRVYSSANNCTFEYVSQPFLMDLEGKQGNFKNLREFVFKNIDGYFKIYSKHTPINLVRDLPQGFSALEPLVDLPIGINITRFQTLLALHRSYLTPGDSSSGWTAGAAAYYVGYLQPRTFLLKYNENGTITDAVDCALDPLSETKCTLKSFTVEKGIYQTSNFRVQPTESIVRFPNITNLCPFGEVFNATRFASVYAWNRKRISNCVADYSVLYNSASFSTFKCYGVSPTKLNDLCFTNVYADSFVIRGDEVRQIAPGQTGKIADYNYKLPDDFTGCVIAWNSNNLDSKVGGNYNYLYRLFRKSNLKPFERDISTEIYQAGSTPCNGVEGFNCYFPLQSYGFQPTNGVGYQPYRVVVLSFELLHAPATVCGPKKSTNLVKNKCVNFNFNGLTGTGVLTESNKKFLPFQQFGRDIADTTDAVRDPQTLEILDITPCSFGGVSVITPGTNTSNQVAVLYQDVNCTEVPVAIHADQLTPTWRVYSTGSNVFQTRAGCLIGAEHVNNSYECDIPIGAGICASYQTQTNSPGSASSVASQSIIAYTMSLGAENSVAYSNNSIAIPTNFTISVTTEILPVSMTKTSVDCTMYICGDSTECSNLLLQYGSFCTQLNRALTGIAVEQDKNTQEVFAQVKQIYKTPPIKDFGGFNFSQILPDPSKPSKRSFIEDLLFNKVTLADAGFIKQYGDCLGDIAARDLICAQKFNGLTVLPPLLTDEMIAQYTSALLAGTITSGWTFGAGAALQIPFAMQMAYRFNGIGVTQNVLYENQKLIANQFNSAIGKIQDSLSSTASALGKLQDVVNQNAQALNTLVKQLSSNFGAISSVLNDILSRLDKVEAEVQIDRLITGRLQSLQTYVTQQLIRAAEIRASANLAATKMSECVLGQSKRVDFCGKGYHLMSFPQSAPHGVVFLHVTYVPAQEKNFTTAPAICHDGKAHFPREGVFVSNGTHWFVTQRNFYEPQIITTDNTFVSGNCDVVIGIVNNTVYDPLQPELDSFKEELDKYFKNHTSPDVDLGDISGINASVVNIQKEIDRLNEVAKNLNESLIDLQELGKYEQGSGYIPEAPRDGQAYVRKDGEWVLLSTFLGSLEHHHHHHHH

SEQ ID NO: 30 - DNA, 2415 bp, Artificial sequence
  hACE2 nucleic acid sequence
atgtcaagctcttcctggctccttctcagccttgttgctgtaactgctgctcagtccaccattgaggaacaggccaagacatttttggacaagtttaaccacgaagccgaagacctgttctatcaaagttcacttgcttcttggaattataacaccaatattactgaagagaatgtccaaaacatgaataatgctggggacaaatggtctgcctttttaaaggaacagtccacacttgcccaaatgtatccactacaagaaattcagaatctcacagtcaagcttcagctgcaggctcttcagcaaaatgggtcttcagtgctctcagaagacaagagcaaacggttgaacacaattctaaatacaatgagcaccatctacagtactggaaaagtttgtaacccagataatccacaagaatgcttattacttgaaccaggtttgaatgaaataatggcaaacagtttagactacaatgagaggctctgggcttgggaaagctggagatctgaggtcggcaagcagctgaggccattatatgaagagtatgtggtcttgaaaaatgagatggcaagagcaaatcattatgaggactatggggattattggagaggagactatgaagtaaatggggtagatggctatgactacagccgcggccagttgattgaagatgtggaacatacctttgaagagattaaaccattatatgaacatcttcatgcctatgtgagggcaaagttgatgaatgcctatccttcctatatcagtccaattggatgcctccctgctcatttgcttggtgatatgtggggtagattttggacaaatctgtactctttgacagttccctttggacagaaaccaaacatagatgttactgatgcaatggtggaccaggcctgggatgcacagagaatattcaaggaggccgagaagttctttgtatctgttggtcttcctaatatgactcaaggattctgggaaaattccatgctaacggacccaggaaatgttcagaaagcagtctgccatcccacagcttgggacctggggaagggcgacttcaggatccttatgtgcacaaaggtgacaatggacgacttcctgacagctcatcatgagatggggcatatccagtatgatatggcatatgctgcacaaccttttctgctaagaaatggagctaatgaaggattccatgaagctgttggggaaatcatgtcactttctgcagccacacctaagcatttaaaatccattggtcttctgtcacccgattttcaagaagacaatgaaacagaaataaacttcctgctcaaacaagcactcacgattgttgggactctgccatttacttacatgttagagaagtggaggtggatggtctttaaaggggaaattcccaaagaccagtggatgaaaaagtggtgggagatgaagcgagagatagttggggtggtggaacctgtgccccatgatgaaacatactgtgaccccgcatctctgttccatgtttctaatgattactcattcattcgatattacacaaggaccctttaccaattccagtttcaagaagcactttgtcaagcagctaaacatgaaggccctctgcacaaatgtgacatctcaaactctacagaagctggacagaaactgttcaatatgctgaggcttggaaaatcagaaccctggaccctagcattggaaaatgttgtaggagcaaagaacatgaatgtaaggccactgctcaactactttgagcccttatttacctggctgaaagaccagaacaagaattcttttgtgggatggagtaccgactggagtccatatgcagaccaaagcatcaaagtgaggataagcctaaaatcagctcttggagataaagcatatgaatggaacgacaatgaaatgtacctgttccgatcatctgttgcatatgctatgaggcagtactttttaaaagtaaaaaatcagatgattctttttggggaggaggatgtgcgagtggctaatttgaaaccaagaatctcctttaatttctttgtcactgcacctaaaaatgtgtctgatatcattcctagaactgaagttgaaaaggccatcaggatgtcccggagccgtatcaatgatgctttccgtctgaatgacaacagcctagagtttctggggatacagccaacacttggacctcctaaccagccccctgtttccatatggctgattgtttttggagttgtgatgggagtgatagtggttggcattgtcatcctgatcttcactgggatcagagatcggaagaagaaaaataaagcaagaagtggagaaaatccttatgcctccatcgatattagcaaaggagaaaataatccaggattccaaaacactgatgatgttcagacctccttt

SEQ ID NO: 31 - DNA, 3183 bp, Artificial sequence
  hACE2mRb3 nucleic acid sequence
atgtcaagctcttcctggctccttctcagccttgttgctgtaactgctgctcagtccaccattgaggaacaggccaagacatttttggacaagtttaaccacgaagccgaagacctgttctatcaaagttcacttgcttcttggaattataacaccaatattactgaagagaatgtccaaaacatgaataatgctggggacaaatggtctgcctttttaaaggaacagtccacacttgcccaaatgtatccactacaagaaattcagaatctcacagtcaagcttcagctgcaggctcttcagcaaaatgggtcttcagtgctctcagaagacaagagcaaacggttgaacacaattctaaatacaatgagcaccatctacagtactggaaaagtttgtaacccagataatccacaagaatgcttattacttgaaccaggtttgaatgaaataatggcaaacagtttagactacaatgagaggctctgggcttgggaaagctggagatctgaggtcggcaagcagctgaggccattatatgaagagtatgtggtcttgaaaaatgagatggcaagagcaaatcattatgaggactatggggattattggagaggagactatgaagtaaatggggtagatggctatgactacagccgcggccagttgattgaagatgtggaacatacctttgaagagattaaaccattatatgaacatcttcatgcctatgtgagggcaaagttgatgaatgcctatccttcctatatcagtccaattggatgcctccctgctcatttgcttggtgatatgtggggtagattttggacaaatctgtactctttgacagttccctttggacagaaaccaaacatagatgttactgatgcaatggtggaccaggcctgggatgcacagagaatattcaaggaggccgagaagttctttgtatctgttggtcttcctaatatgactcaaggattctgggaaaattccatgctaacggacccaggaaatgttcagaaagcagtctgccatcccacagcttgggacctggggaagggcgacttcaggatccttatgtgcacaaaggtgacaatggacgacttcctgacagctcatcatgagatggggcatatccagtatgatatggcatatgctgcacaaccttttctgctaagaaatggagctaatgaaggattccatgaagctgttggggaaatcatgtcactttctgcagccacacctaagcatttaaaatccattggtcttctgtcacccgattttcaagaagacaatgaaacagaaataaacttcctgctcaaacaagcactcacgattgttgggactctgccatttacttacatgttagagaagtggaggtggatggtctttaaaggggaaattcccaaagaccagtggatgaaaaagtggtgggagatgaagcgagagatagttggggtggtggaacctgtgccccatgatgaaacatactgtgaccccgcatctctgttccatgtttctaatgattactcattcattcgatattacacaaggaccctttaccaattccagtttcaagaagcactttgtcaagcagctaaacatgaaggccctctgcacaaatgtgacatctcaaactctacagaagctggacagaaactgttcaatatgctgaggcttggaaaatcagaaccctggaccctagcattggaaaatgttgtaggagcaaagaacatgaatgtaaggccactgctcaactactttgagcccttatttacctggctgaaagaccagaacaagaattcttttgtgggatggagtaccgactggagtccatatgcagaccaaagcatcaaagtgaggataagcctaaaatcagctcttggagataaagcatatgaatggaacgacaatgaaatgtacctgttccgatcatctgttgcatatgctatgaggcagtactttttaaaagtaaaaaatcagatgattctttttggggaggaggatgtgcgagtggctaatttgaaaccaagaatctcctttaatttctttgtcactgcacctaaaaatgtgtctgatatcattcctagaactgaagttgaaaaggccatcaggatgtcccggagccgtatcaatgatgctttccgtctgaatgacaacagcctagagtttctggggatacagccaacacttggacctcctaaccagccccctgtttccatatggctgattgtttttggagttgtgatgggagtgatagtggttggcattgtcatcctgatcttcactgggatcagagatcggaagaagaaaaataaagcaagaagtggagaaaatccttatgcctccatcgatattagcaaaggagaaaataatccaggattccaaaacactgatgatgttcagacctcctttgctagcggcggtggtggcagcggtagcggttctgtgagcaagggcgaggagctgatcaaggagaacatgcgcatgaaggtggtgatggagggcagcgtgaacggccaccagttcaagtgcaccggcgagggcgagggccgcccctacgagggcgtgcagaccatgcgcatcaaggtgatcgagggcggccccctgcccttcgccttcgacatcctggccaccagcttcatgtacggcagccgcaccttcatcaagtaccccgccgacatccccgacttcttcaagcagagcttccccgagggcttcacctgggagcgcgtgacccgctacgaggacggcggcgtggtgaccgtgacccaggacaccagcctggaggacggcgagctggtgtacaacgtgaaggtgcgcggcgtgaacttccccagcaacggccccgtgatgcagaagaagaccaagggctgggagcccaacaccgagatgatgtaccccgccgacggcggcctgcgcggctacaccgacatcgccctgaaggtggacggcggcggccacctgcactgcaacttcgtgaccacctaccgcagcaagaagaccgtgggcaacatcaagatgcccggcgtgcacgccgtggaccaccgcctggagcgcatcgaggagagcgacaacgagacctacgtggtgcagcgcgaggtggccgtggccaagtacagcaacctgggcggcggcatggacgagctgtacaagggatcccaccaccaccaccaccactaa

SEQ ID NO: 32 - protein, 1060 aa, Artificial sequence
  hACE2mRb3 amino acid sequence
MSSSSWLLLSLVAVTAAQSTIEEQAKTFLDKFNHEAEDLFYQSSLASWNYNTNITEENVQNMNNAGDKWSAFLKEQSTLAQMYPLQEIQNLTVKLQLQALQQNGSSVLSEDKSKRLNTILNTMSTIYSTGKVCNPDNPQECLLLEPGLNEIMANSLDYNERLWAWESWRSEVGKQLRPLYEEYVVLKNEMARANHYEDYGDYWRGDYEVNGVDGYDYSRGQLIEDVEHTFEEIKPLYEHLHAYVRAKLMNAYPSYISPIGCLPAHLLGDMWGRFWTNLYSLTVPFGQKPNIDVTDAMVDQAWDAQRIFKEAEKFFVSVGLPNMTQGFWENSMLTDPGNVQKAVCHPTAWDLGKGDFRILMCTKVTMDDFLTAHHEMGHIQYDMAYAAQPFLLRNGANEGFHEAVGEIMSLSAATPKHLKSIGLLSPDFQEDNETEINFLLKQALTIVGTLPFTYMLEKWRWMVFKGEIPKDQWMKKWWEMKREIVGVVEPVPHDETYCDPASLFHVSNDYSFIRYYTRTLYQFQFQEALCQAAKHEGPLHKCDISNSTEAGQKLFNMLRLGKSEPWTLALENVVGAKNMNVRPLLNYFEPLFTWLKDQNKNSFVGWSTDWSPYADQSIKVRISLKSALGDKAYEWNDNEMYLFRSSVAYAMRQYFLKVKNQMILFGEEDVRVANLKPRISFNFFVTAPKNVSDIIPRTEVEKAIRMSRSRINDAFRLNDNSLEFLGIQPTLGPPNQPPVSIWLIVFGVVMGVIVVGIVILIFTGIRDRKKKNKARSGENPYASIDISKGENNPGFQNTDDVQTSFASGGGGSGSGSVSKGEELIKENMRMKVVMEGSVNGHQFKCTGEGEGRPYEGVQTMRIKVIEGGPLPFAFDILATSFMYGSRTFIKYPADIPDFFKQSFPEGFTWERVTRYEDGGVVTVTQDTSLEDGELVYNVKVRGVNFPSNGPVMQKKTKGWEPNTEMMYPADGGLRGYTDIALKVDGGGHLHCNFVTTYRSKKTVGNIKMPGVHAVDHRLERIEESDNETYVVQREVAVAKYSNLGGGMDELYKGSHHHHHH

SEQ ID NO: 33 - protein, 1483 aa, Artificial sequence
  SARS-CoV2-SMG amino acid sequence
MARSVTLVFLVLVSLTGLYAVNLTTRTQLPPAYTNSFTRGVYYPDKVFRSSVLHSTQDLFLPFFSNVTWFHAIHVSGTNGTKRFDNPVLPFNDGVYFASTEKSNIIRGWIFGTTLDSKTQSLLIVNNATNVVIKVCEFQFCNDPFLGVYYHKNNKSWMESEFRVYSSANNCTFEYVSQPFLMDLEGKQGNFKNLREFVFKNIDGYFKIYSKHTPINLVRDLPQGFSALEPLVDLPIGINITRFQTLLALHRSYLTPGDSSSGWTAGAAAYYVGYLQPRTFLLKYNENGTITDAVDCALDPLSETKCTLKSFTVEKGIYQTSNFRVQPTESIVRFPNITNLCPFGEVFNATRFASVYAWNRKRISNCVADYSVLYNSASFSTFKCYGVSPTKLNDLCFTNVYADSFVIRGDEVRQIAPGQTGKIADYNYKLPDDFTGCVIAWNSNNLDSKVGGNYNYLYRLFRKSNLKPFERDISTEIYQAGSTPCNGVEGFNCYFPLQSYGFQPTNGVGYQPYRVVVLSFELLHAPATVCGPKKSTNLVKNKCVNFNFNGLTGTGVLTESNKKFLPFQQFGRDIADTTDAVRDPQTLEILDITPCSFGGVSVITPGTNTSNQVAVLYQDVNCTEVPVAIHADQLTPTWRVYSTGSNVFQTRAGCLIGAEHVNNSYECDIPIGAGICASYQTQTNSPGSASSVASQSIIAYTMSLGAENSVAYSNNSIAIPTNFTISVTTEILPVSMTKTSVDCTMYICGDSTECSNLLLQYGSFCTQLNRALTGIAVEQDKNTQEVFAQVKQIYKTPPIKDFGGFNFSQILPDPSKPSKRSFIEDLLFNKVTLADAGFIKQYGDCLGDIAARDLICAQKFNGLTVLPPLLTDEMIAQYTSALLAGTITSGWTFGAGAALQIPFAMQMAYRFNGIGVTQNVLYENQKLIANQFNSAIGKIQDSLSSTASALGKLQDVVNQNAQALNTLVKQLSSNFGAISSVLNDILSRLDKVEAEVQIDRLITGRLQSLQTYVTQQLIRAAEIRASANLAATKMSECVLGQSKRVDFCGKGYHLMSFPQSAPHGVVFLHVTYVPAQEKNFTTAPAICHDGKAHFPREGVFVSNGTHWFVTQRNFYEPQIITTDNTFVSGNCDVVIGIVNNTVYDPLQPELDSFKEELDKYFKNHTSPDVDLGDISGINASVVNIQKEIDRLNEVAKNLNESLIDLQELGKYEFGGGGSGGGGSGGGGSGGGGSGVSKGEEASGRALFQYPMTSKIELNGEINGKKFKVAGEGFTPSSGRFNMHAYCTTGDLPMSWVVIASPLQYGFHMFAHYPEDITHFFQECFPGSYTLDRTLRMEGDGTLTTHHEYSLEDGCVTSKTTLNASGFDPKGATMTKSFVKQLPNEVKITPHGPNGIRLTSTVLYLKEDGTIQIGTQDCIVTPVGGRKVTQPKAHFLHTQIIQKKDPNDTRDHIVQTELAVAGNLWHGMDELYKSLEHHHHHHHH

SEQ ID NO: 34 - DNA, 4452 bp, Artificial sequence
  SARS-CoV2-SMG nucleic acid sequence
atggcccgcagcgtgaccctggtgttcctggtgctggtgagcctgaccggtctgtacgccgtgaacctgaccacccgcacccagctgccccccgcctacaccaacagcttcacccgcggcgtgtactaccccgacaaggtgttccgcagcagcgtgctgcacagcacccaggacctgttcctgcccttcttcagcaacgtgacctggttccacgccatccacgtgagcggcaccaacggcaccaagcgcttcgacaaccccgtgctgcccttcaacgacggcgtgtacttcgccagcaccgagaagagcaacatcatccgcggctggatcttcggcaccaccctggacagcaagacccagagcctgctgatcgtgaacaacgccaccaacgtggtgatcaaggtgtgcgagttccagttctgcaacgaccccttcctgggcgtgtactaccacaagaacaacaagagctggatggagagcgagttccgcgtgtacagcagcgccaacaactgcaccttcgagtacgtgagccagcccttcctgatggacctggagggcaagcagggcaacttcaagaacctgcgcgagttcgtgttcaagaacatcgacggctacttcaagatatacagcaagcacacccccatcaacctggtgcgcgacctgccccagggcttcagcgccctggagcccctggtggacctgcccatcggcatcaacatcacccgcttccagaccctgctggccctgcaccgcagctacctgacccccggcgacagcagcagcggctggaccgccggcgccgccgcctactacgtgggctacctgcagccccgcaccttcctgctgaagtacaacgagaacggcaccatcaccgacgccgtggactgcgccctggaccccctgagcgagaccaagtgcaccctgaagagcttcaccgtggagaagggcatctaccagaccagcaacttccgcgtgcagcccaccgagagcatcgtgcgcttccccaacatcaccaacctgtgccccttcggcgaggtgttcaacgccacccgcttcgccagcgtgtacgcctggaaccgcaagcgcatcagcaactgcgtggccgactacagcgtgctgtacaacagcgccagcttcagcaccttcaagtgctacggcgtgagccccaccaagctgaacgacctgtgcttcaccaacgtgtacgccgacagcttcgtgatccgcggcgacgaggtgcgccagatcgcccccggccagaccggcaagatcgccgactacaactacaagctgcccgacgacttcaccggctgcgtgatcgcctggaacagcaacaacctggacagcaaggtgggcggcaactacaactacctgtaccgcctgttccgcaagagcaacctgaagcccttcgagcgcgacatcagcaccgagatataccaggccggcagcaccccctgcaacggcgtggagggcttcaactgctacttccccctgcagagctacggcttccagcccaccaacggcgtgggctaccagccctaccgcgtggtggtgctgagcttcgagctgctgcacgcccccgccaccgtgtgcggccccaagaagagcaccaacctggtgaagaacaagtgcgtgaacttcaacttcaacggcctgaccggcaccggcgtgctgaccgagagcaacaagaagttcctgcccttccagcagttcggccgcgacatcgccgacaccaccgacgccgtgcgcgacccccagaccctggagatcctggacatcaccccctgcagcttcggcggcgtgagcgtgatcacccccggcaccaacaccagcaaccaggtggccgtgctgtaccaggacgtgaactgcaccgaggtgcccgtggccatccacgccgaccagctgacccccacctggcgcgtgtacagcaccggcagcaacgtgttccagacccgcgccggctgcctgatcggcgccgagcacgtgaacaacagctacgagtgcgacatccccatcggcgccggcatctgcgccagctaccagacccagaccaacagccccggtagcgcgagctctgtggccagccagagcatcatcgcctacaccatgagcctgggcgccgagaacagcgtggcctacagcaacaacagcatcgccatccccaccaacttcaccatcagcgtgaccaccgagatcctgcccgtgagcatgaccaagaccagcgtggactgcaccatgtacatctgcggcgacagcaccgagtgcagcaacctgctgctgcagtacggcagcttctgcacccagctgaaccgcgccctgaccggcatcgccgtggagcaggacaagaacacccaggaggtgttcgcccaggtgaagcagatatacaagaccccccccatcaaggacttcggcggcttcaacttcagccagatcctgcccgaccccagcaagcccagcaagcgcagcttcatcgaggacctgctgttcaacaaggtgaccctggccgacgccggcttcatcaagcagtacggcgactgcctgggcgacatcgccgcccgcgacctgatctgcgcccagaagttcaacggcctgaccgtgctgccccccctgctgaccgacgagatgatcgcccagtacaccagcgccctgctggccggcaccatcaccagcggctggaccttcggcgccggcgccgccctgcagatccccttcgccatgcagatggcctaccgcttcaacggcatcggcgtgacccagaacgtgctgtacgagaaccagaagctgatcgccaaccagttcaacagcgccatcggcaagatccaggacagcctgagcagcaccgccagcgccctgggcaagctgcaggacgtggtgaaccagaacgcccaggccctgaacaccctggtgaagcagctgagcagcaacttcggcgccatcagcagcgtgctgaacgacatcctgagccgcctggacaaggtggaggccgaggtgcagatcgaccgcctgatcaccggccgcctgcagagcctgcagacctacgtgacccagcagctgatccgcgccgccgagatccgcgccagcgccaacctggccgccaccaagatgagcgagtgcgtgctgggccagagcaagcgcgtggacttctgcggcaagggctaccacctgatgagcttcccccagagcgccccccacggcgtggtgttcctgcacgtgacctacgtgcccgcccaggagaagaacttcaccaccgcccccgccatctgccacgacggcaaggcccacttcccccgcgagggcgtgttcgtgagcaacggcacccactggttcgtgacccagcgcaacttctacgagccccagatcatcaccaccgacaacaccttcgtgagcggcaactgcgacgtggtgatcggcatcgtgaacaacaccgtgtacgaccccctgcagcccgagctggacagcttcaaggaggagctggacaagtacttcaagaaccacaccagccccgacgtggacctgggcgacatcagcggcatcaacgctagcgtggtgaacatccagaaggagatcgaccgcctgaacgaggtggccaagaacctgaacgagagcctgatcgacctgcaggagctgggcaagtacgaattcggcggcggaggaagcggaggaggtggcagcggtggcggtggctccggcggaggtggatccggcgtgagcaagggcgaggaggcatctggcagagccctgttccagtaccccatgaccagcaagatcgagctgaacggcgagatcaacggcaagaaattcaaggtggccggcgagggcttcacccccagcagcggcagattcaacatgcacgcctactgcaccaccggcgacctgcctatgagctgggtcgtgattgccagccccctccagtacggcttccacatgttcgcccactaccccgaggacatcacacactttttccaggaatgcttccccggcagctacaccctggaccggaccctgagaatggaaggcgacggcaccctgaccacccaccacgagtacagcctggaggacggctgcgtgacctccaagaccaccctgaatgccagcggcttcgaccctaagggcgccaccatgaccaagagcttcgtgaaacaactgcctaacgaggtgaagatcaccccccacggccccaacggcatcagactgaccagcaccgtgctgtacctgaaggaggatggcaccatccagatcggcacccaggactgcatcgtgacccctgtgggcggaaggaaagtgacccagcccaaggcccacttcctgcacacccagatcatccagaagaaggaccccaacgacacccgggaccacatcgtgcagacagaactggccgtggccggcaatctgtggcacggcatggacgagctgtacaagagcctcgagcatcaccaccaccaccaccaccactaa

SEQ ID NO: 35 - protein, 699 aa, Artificial sequence
  SARS-CoV2-S1 amino acid sequence
MARSVTLVFLVLVSLTGLYAVNLTTRTQLPPAYTNSFTRGVYYPDKVFRSSVLHSTQDLFLPFFSNVTWFHAIHVSGTNGTKRFDNPVLPFNDGVYFASTEKSNIIRGWIFGTTLDSKTQSLLIVNNATNVVIKVCEFQFCNDPFLGVYYHKNNKSWMESEFRVYSSANNCTFEYVSQPFLMDLEGKQGNFKNLREFVFKNIDGYFKIYSKHTPINLVRDLPQGFSALEPLVDLPIGINITRFQTLLALHRSYLTPGDSSSGWTAGAAAYYVGYLQPRTFLLKYNENGTITDAVDCALDPLSETKCTLKSFTVEKGIYQTSNFRVQPTESIVRFPNITNLCPFGEVFNATRFASVYAWNRKRISNCVADYSVLYNSASFSTFKCYGVSPTKLNDLCFTNVYADSFVIRGDEVRQIAPGQTGKIADYNYKLPDDFTGCVIAWNSNNLDSKVGGNYNYLYRLFRKSNLKPFERDISTEIYQAGSTPCNGVEGFNCYFPLQSYGFQPTNGVGYQPYRVVVLSFELLHAPATVCGPKKSTNLVKNKCVNFNFNGLTGTGVLTESNKKFLPFQQFGRDIADTTDAVRDPQTLEILDITPCSFGGVSVITPGTNTSNQVAVLYQDVNCTEVPVAIHADQLTPTWRVYSTGSNVFQTRAGCLIGAEHVNNSYECDIPIGAGICASYQTQTNSPRRGGGGSHHHHHH

SEQ ID NO: 36 - DNA, 2100 bp, Artificial sequence
  SARS-CoV2-S1 nucleic acid sequence
atggcccgcagcgtgaccctggtgttcctggtgctggtgagcctgaccggtctgtacgccgtgaacctgaccacccgcacccagctgccccccgcctacaccaacagcttcacccgcggcgtgtactaccccgacaaggtgttccgcagcagcgtgctgcacagcacccaggacctgttcctgcccttcttcagcaacgtgacctggttccacgccatccacgtgagcggcaccaacggcaccaagcgcttcgacaaccccgtgctgcccttcaacgacggcgtgtacttcgccagcaccgagaagagcaacatcatccgcggctggatcttcggcaccaccctggacagcaagacccagagcctgctgatcgtgaacaacgccaccaacgtggtgatcaaggtgtgcgagttccagttctgcaacgaccccttcctgggcgtgtactaccacaagaacaacaagagctggatggagagcgagttccgcgtgtacagcagcgccaacaactgcaccttcgagtacgtgagccagcccttcctgatggacctggagggcaagcagggcaacttcaagaacctgcgcgagttcgtgttcaagaacatcgacggctacttcaagatatacagcaagcacacccccatcaacctggtgcgcgacctgccccagggcttcagcgccctggagcccctggtggacctgcccatcggcatcaacatcacccgcttccagaccctgctggccctgcaccgcagctacctgacccccggcgacagcagcagcggctggaccgccggcgccgccgcctactacgtgggctacctgcagccccgcaccttcctgctgaagtacaacgagaacggcaccatcaccgacgccgtggactgcgccctggaccccctgagcgagaccaagtgcaccctgaagagcttcaccgtggagaagggcatctaccagaccagcaacttccgcgtgcagcccaccgagagcatcgtgcgcttccccaacatcaccaacctgtgccccttcggcgaggtgttcaacgccacccgcttcgccagcgtgtacgcctggaaccgcaagcgcatcagcaactgcgtggccgactacagcgtgctgtacaacagcgccagcttcagcaccttcaagtgctacggcgtgagccccaccaagctgaacgacctgtgcttcaccaacgtgtacgccgacagcttcgtgatccgcggcgacgaggtgcgccagatcgcccccggccagaccggcaagatcgccgactacaactacaagctgcccgacgacttcaccggctgcgtgatcgcctggaacagcaacaacctggacagcaaggtgggcggcaactacaactacctgtaccgcctgttccgcaagagcaacctgaagcccttcgagcgcgacatcagcaccgagatataccaggccggcagcaccccctgcaacggcgtggagggcttcaactgctacttccccctgcagagctacggcttccagcccaccaacggcgtgggctaccagccctaccgcgtggtggtgctgagcttcgagctgctgcacgcccccgccaccgtgtgcggccccaagaagagcaccaacctggtgaagaacaagtgcgtgaacttcaacttcaacggcctgaccggcaccggcgtgctgaccgagagcaacaagaagttcctgcccttccagcagttcggccgcgacatcgccgacaccaccgacgccgtgcgcgacccccagaccctggagatcctggacatcaccccctgcagcttcggcggcgtgagcgtgatcacccccggcaccaacaccagcaaccaggtggccgtgctgtaccaggacgtgaactgcaccgaggtgcccgtggccatccacgccgaccagctgacccccacctggcgcgtgtacagcaccggcagcaacgtgttccagacccgcgccggctgcctgatcggcgccgagcacgtgaacaacagctacgagtgcgacatccccatcggcgccggcatctgcgccagctaccagacccagaccaacagcccccgccgcggtggcggtggatcccaccaccaccaccaccactaa

SEQ ID NO: 37 - protein, 20 aa, Artificial sequence
  B2M signal peptide amino acid sequence
MARSVTLVFLVLVSLTGLYA

SEQ ID NO: 38 - protein, 238 aa, Artificial sequence
  Green fluorescent protein mGamillus amino acid sequence
VSKGEEASGRALFQYPMTSKIELNGEINGKKFKVAGEGFTPSSGRFNMHAYCTTGDLPMSWVVIASPLQYGFHMFAHYPEDITHFFQECFPGSYTLDRTLRMEGDGTLTTHHEYSLEDGCVTSKTTLNASGFDPKGATMTKSFVKQLPNEVKITPHGPNGIRLTSTVLYLKEDGTIQIGTQDCIVTPVGGRKVTQPKAHFLHTQIIQKKDPNDTRDHIVQTELAVAGNLWHGMDELYK

SEQ ID NO: 39 - protein, 235 aa, Artificial sequence
  Green fluorescent protein mNeonGreen amino acid sequence
VSKGEEDNMASLPATHELHIFGSINGVDFDMVGQGTGNPNDGYEELNLKSTKGDLQFSPWILVPHIGYGFHQYLPYPDGMSPFQAAMVDGSGYQVHRTMQFEDGASLTVNYRYTYEGSHIKGEAQVKGTGFPADGPVMTNSLTAADWCRSKKTYPNDKTIISTFKWSYTTGNGKRYRSTARTTYTFAKPMAANYLKNQPMYVFRKTELKHSKTELNFKEWQKAFTDVMGMDELYK

SEQ ID NO: 40 - protein, 27 aa, Artificial sequence
  TFD amino acid sequence
YIPEAPRDGQAYVRKDGEWVLLSTFLG

SEQ ID NO: 41 - protein, 805 aa, Artificial sequence [sequence omitted]

SEQ ID NO: 42 - protein, 236 aa, Artificial sequence
  Red fluorescent protein mRuby3 amino acid sequence
VSKGEELIKENMRMKVVMEGSVNGHQFKCTGEGEGRPYEGVQTMRIKVIEGGPLPFAFDILATSFMYGSRTFIKYPADIPDFFKQSFPEGFTWERVTRYEDGGVVTVTQDTSLEDGELVYNVKVRGVNFPSNGPVMQKKTKGWEPNTEMMYPADGGLRGYTDIALKVDGGGHLHCNFVTTYRSKKTVGNIKMPGVHAVDHRLERIEESDNETYVVQREVAVAKYSNLGGGMDELYK